European Patent Application EP 4 721 566 A1, published April 8, 2026. Title: Microbial compostion based on Bacillus infantis strain for agricultural use. Applicant: Kimitec Biogroup. Application EP. The sequence listing filed with the application follows.

SEQUENCE LISTING (8 sequences)

SEQ ID NO: 1 - DNA, 1430 bp, Bacillus subtilis
  source 1..1430: mol_type = genomic DNA
cttaggcggctggctccaaaaggttaccccaccgacttcgggtgttacaaactctcgtggtgtgacgggcggtgtgtacaaggcccgggaacgtattcaccgcggcatgctgatccgcgattactagcgattccagcttcatgcaggcgagttgcagcctgcaatccgaactgagaatggttttatgggattcgcttaacctcgcggtcttgcagccctttgtaccatccattgtagcacgtgtgtagcccaggtcataaggggcatgatgatttgacgtcatccccaccttcctccggtttgtcaccggcagtcaccttagagtgcccaactgaatgctggcaactaagatcaagggttgcgctcgttgcgggacttaacccaacatctcacgacacgagctgacgacaaccatgcaccacctgtcatcctgtcccccgaaggggaacgccctatctctagggttgtcaggagatgtcaagacctggtaaggttcttcgcgttgcttcgaattaaaccacatgctccaccgcttgtgcgggcccccgtcaattcctttgagtttcagccttgcggccgtactccccaggcggagtgcttaatgcgtttgctgcagcactaaagggcggaaaccctctaacacttagcactcatcgtttacggcgtggactaccagggtatctaatcctgtttgctccccacgctttcgcgcctcagcgtcagttacagaccagaaagtcgccttcgccactggtgttcctccacatctctacgcatttcaccgctacacgtggaattccactttcctcttctgcactcaagtcccccagtttccaatgaccctccacggttgagccgtgggctttcacatcagacttaagagaccgcctgcgcgcgctttacgcccaataattccggacaacgcttgccacctacgtattaccgcggctgctggcacgtagttagccgtggctttctggtcaggtaccgtcaaggtgccggcagttactccggcacttgttcttccctgacaacagagttttacgatccgaaaaccttcatcactcacgcggcgttgctccgtcagactttcgtccattgcggaagattccctactgctgcctcccgtaggagtctgggccgtgtctcagtcccagtgtggccgatcaccctctcaggtcggctacgcatcgttgccttggtgagccgttacctcaccaactagctaatgcgccgcgggcccatctgtaagtgatagccgaaaccatctttcagcatagcctcatgagaggctgtgcattatccggtattagctccggtttcccgaagttatcccagtcttacaggcaggttgcccacgtgttactcacccgtccgccgctgacttcagggagcaagctcccatccgtccgctcgactgcatgtatagc

SEQ ID NO: 2 - DNA, 1366 bp, Bacillus subtilis
  source 1..1366: mol_type = genomic DNA
ctccaaactccctaactttatgtaggatttcggaagggggcacactccatgtgcttacctgctcaccttttattccgtacgccttgccggtttcctgttgaagcggttcgcttaataaaaaagaaggatattccctaaaagaaccaaacctgcttcaaccgtttgcatgcggttttgcttttttgactgcattttatttcgataggtgcgctggagctttctaaagataaattcctttttcattttatcgctccttattttccgcttctatacacctttgcctgttctattgcaaatgctaacgcctctcttgaaaataaatatttaagaagctcatcataagtgctagtttgaaagataagctctttatcattaaaaatataaattgcaggaccggttagctgttctccattattcaatttgagagattcttgagttgttatagaaccggccaatttcaagtcttctttgtgtggtgttttaagcggttgaagaaatttagaatctccaatggcaaggattgaccatttgccaggtttcttggaaagccactttgggtcattaagtatttgatcactgtccctcaatacttgtaattcttcaatcactggactgtaaaactttgaaataaggtctcttgcttttacactaacttcctggccagttctgaccagcaggtcaggctcaataatgagctgccttccatttatagtgacaaatcccaaatcgtgatctatttctgatactgttccttctataacctctttgaatataatattttccctgatatattttttcatagttactacgtcatctgtgcgtacgatctccttttggtggtcaaaaagtaagaaggctttactattgtcaatttttaattcaggcaataattgtttgtcagctttgttataaaagattagcatattagaaaattcggtttgcaaatcaagctgtgcacgttcggcagattgagtgtcctcatcaacaatgagaatggaataggttccaaaatatctagcataatattcttttaatttgacttcgctcgtttttaaaggaattatataatcagctctctttccatctttccaatatgcctttatgttaatagtcgacaggccagtagcatttggcatataatggttgattttactatcagtagtgccaataaatttgccattataatcctgagaacctttattaaaataaatcggctcctccccttccggaaactcaatcctcatttcctcattcaccggcacctcctgatatttcaaagatttagagatatccttcatctctttctccaccagtccggcattccaccggtaagaacccatgattgcctgcacctctgtatctccat

SEQ ID NO: 3 - DNA, 1249 bp, Bacillus subtilis
  source 1..1249: mol_type = genomic DNA
tcttatttacgtaatcccacctaataaaaatttataagaggtcccttggcttcttttgtggctgggctgggaacctgtctctgttaatctctataccctcggggaggggaatctattactttatgataacattcattgacatgaaagagccaaggggacagaccccttggctctttctgatggtgggccaaggggtctgtcccccgggctcatattattttgcttcaatttcttctaattcagaccaaacttcagtaaatggataaaagctgcagctgaatttaaatggatgttctaagtcgtaaatattttcccattccccatcaattaatttttgatcatataggctataaaatgcatcgatttgataacaggcattatccgtaactttttctatatactctgattgcacctcattcaaatttgaagtaccgacattttctaaatcttctaccgttgttgggtaaccgatagtagtcaatagttccgcaacaaattgtttatcttcatctgctaaaacactttcagcttcaaattcgatactattcaggtaatgatttggaaattcttgttccataatttcaaaacggtaatcactgcttccataaaaattcaaataaacagaggccccactactcgtatcaatagcaaatcgctctttgtcatacgtatcttcacttattagtacgttaaagtcatttttatattttttataaaagtccgtctgttccaaatcctgtatagagaatagttttggttctaaggttggacgcattgaaactatgtaatctaaatacaaaccatttaattcttcgtgttttctttcttcaaaaaaaccggatacgatactaaaaatcttaaatatcaacacaaaaaaaagaataagaattactccaaaacacccactgccatgattgttattttttttcacgtaatccactccataaattattctaatattaatatcggaacatttaagagtgtattaataacggatgaagccaaggggtctgtcccctggctccttttgtggctgggctggggatctgtctctgttattctctttaccctcttggaggggaatctattacactatgataacatccattgagatgtatcgcctttgacatgatatttatcgctaaataggttcaatattgaaaaacgtagtagattcatattttgcagtaagacttttatgtttttcgaactttgtgtaggaatacttaaagtaacggagaggttagtt

SEQ ID NO: 4 - DNA, 1067 bp, Bacillus subtilis
  source 1..1067: mol_type = genomic DNA
caagaaaggttacaattaattttaaacaaaggatacctgctccttttataaaataaaaaagccgccagttttggcagcgatttggaatttaagctcccggtagctgaagatgtcatctcagttttcactgaaatacatatcggcataataatcaatttccttgtccttccgtataattgatatcatttcttcaaccactacagaagaaagtattccttcttcattgaaatgatgagcaaaattgactgctaactgtttgatatcaataacaggattttgaaggagaacaaccaagctttgttcaatcaaatgttcatttcccttagtattttcataaagatagttcaaagcgagggtaatctcttgctcgttagtcgttgataaggctgtgttaagttcatcgggggtccaatgtcttccctcttgttcaagataaatatcttcaagttctgctttttctacgtataatccatttaagaatatgtcaaaattaggagctaattcaataatctgttcagattccatatcaatgtatattaccggaggctctacttttgtatttctgtaatctaatgctacccacgaatgcccacttcctgagactaaaacaatatttttcggcaaaccccattcttttattaagtattcactttctaatatacctttttcttcacctatacctaaaatgtgatcaatattaatatgatcatcagcccaagatgttgggacattagaagggaacgaattatagttaatatatccaccattctggatcttaagaagataaatataggatttaggcaacttcactttaagttttttttctgctctttctacttctttatcttttaaaggttccaatttatagtattcatcatcttcttgccatatctttttcacagcggcattctctcccaaaaaactcttttattagttagaacttcaaaataattatttggcaatttctattaagcttaaatgctcctttctccacaaaaggaagcagactggatgaattaaagatttcccataggaaaactcatacagatatctccccaatcatccat

SEQ ID NO: 5 - DNA, 840 bp, Bacillus subtilis
  source 1..840: mol_type = genomic DNA
cttggagaggatgctattaactttttcaattatctgagcggctatatggagaggccatcctatcaacagttatctgtttcacctttcggcatcagagatactttcatcaggctcatcgatcaggagatagaatttcacaggaactatcagaatggaagaatcatagcaaaaatgaattctctgactgacaagaaaatcattaaaaaattgtatgaagcctcgatagcaggggttaagatagatcttatcatcaggggggtctgctgcttaaggcccggcattgcgggtgtcagtgaaaacatcaaggtccttagcattgtgggtacattccttgaacacaccagaatcttttatttcgatcatcagcaagctaaaagggtttacctttcttcggcagactggatgacccgtaatatggaaaaccgtgttgagattctttttcccattctggaggagcggcttaaagcaagggtttatagtgtacttgaggttatgctgaaagataactgcaaagcaagggaacaggaccatgatggccgttatcgctatgtggaccggaaaagcggcgaaaaccgtataaacagccagcagctgttatgtgaagaagctgtccagtttaagctttcgtcgaagactgcagacagctatcctcctgcacatcgtccacgaccggcttcacttgcagaatcttacttactgaagctgaaggagtttattccattgcttaacagatagaaaagattcaccattcatacatgaataaggcagtcgtttccccctcagggtcctataataaagatggaaaaaaacttccagcgggggggatttttatgcgttatg

SEQ ID NO: 6 - DNA, 838 bp, Bacillus subtilis
  source 1..838: mol_type = genomic DNA
cttaccgaagccgggctggaggagctgatgagagaaggggaggcgccttccggcagtcatgagggacatcattaagaagtgaaggaaaaagatccgttgaaaagttcaatgggtctttttttgaatagagaatttcaccattcattctagaatagatgaattgacaattttatggtaaaatatcctgaaggaggcgggattcatgaccttttataaagtattatataggatatctcgtttttgtcctgctattgctgatggtttatgttatgattccagctgaatacggcttttatgctcttatgggattaaccatactgttttgcctgtatcaattcatgattttgcggaagaaaagcaagagtacaaagaataattagcagattggtaatttggctgccttactcatttaatggggggcagctatttttatgctgaagtggtgagcggcactgacctccagcacttccattccttagtaaggctctctgaatgagtattcaggtcggcgatcacttcatcaatagctgctgatcgctctccccagcctcgctatcccttcttcaatcctatcaggcatcatactgccgtacccgagaacgatcttatttttgtgattgcctttcatgatgctataatcctcaacaggatatatccggacagaatggctggaaatccagttcagcagcccttcatcaaaaacaatggaggggaactcagcaaccaggtgcatccctgccgcatgaccccagatcctgcagtcaggaaaatggtttttcaagctgtccaccaaagcctgccgacgctgcctgtaaattcttttcatcttccttatatg

SEQ ID NO: 7 - DNA, 495 bp, Bacillus subtilis
  source 1..495: mol_type = genomic DNA
cgcagggaaattgaggagatgaagaagctgattgaggatctggaagaacaggagtagaggcacagcctagatgagaaagaaaagccagacagagggccagtaaatctggccctctgtatttttctgaaaatttataattcatcgttttttctcttgtttccggcagtcataaattatatcctagtctgtatagcattttgcccccggcctgtcttgccactttttcattctatacataaataaggccgggccaatacaagaggagagatgcccatggagaagaagctggcgaataaggtattgattgcgagtctgatagggagttcgattgagtggttcgattattttttatacgggacggtggcagcgcttgtttttaatcaggtgattttccacagtgaggatccggcggtcggcctgctgctcgcgtatgcgtcatttgcgctcgcatttttcatccgtccgctgggcggtgtgacttttgcccatatcggc

SEQ ID NO: 8 - DNA, 640 bp, Bacillus subtilis
  source 1..640: mol_type = genomic DNA
taccatattgatgaacggtgattcaatcttgaagggccagcttccgcatatcccgacgaaatacctagcgttcctcccgccgtgccaggcaccgcaaaaagacagtatccggccttttgtccacgaagggtgccagacacggtgaaacaaaatggctgctcgttcgtatataatgacaaggaagattatgtaatcacaactcttacatccctgctggtaatcatgaaagaggtgaacgcctatgccaacctttcttgttgttaacctttgcattgttttagttctgtctgctattatgtcctatattaagaagaatggagaaaagaaggacaagggatttgttttgtcttactatcaattgagccatagaagaaaaatgattcgctccttatgggagctccctttcctcattctcttcctgatcctgatgttttatctcacggatcttgaaactatctatatgctgtcactttccgccctgctgttcttcgtgttcattggccagttctgctataactactataagtggaagcagcaggaaaaggcatgatcggctgagatcatgccttttcctcattcagcgtgcctggcaccgcaaaaagacaactacccgctatttgtccacagacggtgcctggca